European Patent Application EP 4 729 617 A1, published April 22, 2026. Title: CD25를 표적으로 하는 압타머, 이를 포함하는 약물 접합체, 및 이의 용도. Applicant: 주식회사 압타머사이언스. The sequence listing filed with the application follows.

SEQUENCE LISTING (27 sequences)

SEQ ID NO: 1 - DNA, 43 bp, synthetic construct
  source 1..43: mol_type = other DNA
ttcgagatcaagttatagcgtgtcccattctatccaagacact

SEQ ID NO: 2 - DNA, 40 bp, synthetic construct
  source 1..40: mol_type = other DNA
gtgtgtgtcactctatcgttacgaggaatacgggcaaagc

SEQ ID NO: 3 - DNA, 40 bp, synthetic construct
  source 1..40: mol_type = other DNA
cggtgcaatcgcgtggtcaacatcctgttaacctcggaat

SEQ ID NO: 4 - DNA, 50 bp, synthetic construct
  source 1..50: mol_type = other DNA
  modified_base order(7,9,11,13,17,19,21,24,25,34): mod_base = OTHER; note = thymine or uracil substituted with NapdU(5-naphthylmethylaminocarbonyl-dU)
agttcgtgtgtgtcactctatcgttacgaggaatacgggcaaagcgacca

SEQ ID NO: 5 - DNA, 50 bp, synthetic construct
  source 1..50: mol_type = other DNA
  modified_base order(9,14,19,22,28,31,33,34,39,45): mod_base = OTHER; note = 9,14,19,22,28,31,33,34,39,45
agttccggtgcaatcgcgtggtcaacatcctgttaacctcggaatgacca

SEQ ID NO: 6 - DNA, 50 bp, synthetic construct
  source 1..50: mol_type = other DNA
  modified_base order(10,15,16,18,23,25,30,31,33,35,45): mod_base = OTHER; note = thymine or uracil substituted with NapdU(5-naphthylmethylaminocarbonyl-dU)
agttcgagatcaagttatagcgtgtcccattctatccaagacactgacca

SEQ ID NO: 7 - DNA, 27 bp, synthetic construct
  source 1..27: mol_type = other DNA
ggagttcgtgtgtgtcactctatcgtt

SEQ ID NO: 8 - DNA, 22 bp, synthetic construct
  source 1..22: mol_type = other DNA
gtcgctttgcccgtattcctcg

SEQ ID NO: 9 - DNA, 19 bp, synthetic construct
  source 1..19: mol_type = other DNA
gttccggtgcaatcgcgtg

SEQ ID NO: 10 - DNA, 25 bp, synthetic construct
  source 1..25: mol_type = other DNA
ggaggtcattccgaggttaacagga

SEQ ID NO: 11 - DNA, 29 bp, synthetic construct
  source 1..29: mol_type = other DNA
ggagttcgagatcaagttatagcgtgtcc

SEQ ID NO: 12 - DNA, 27 bp, synthetic construct
  source 1..27: mol_type = other DNA
ggaggtcagtgtcttggatagaatggg

SEQ ID NO: 13 - DNA, 27 bp, synthetic construct
  source 1..27: mol_type = other DNA
  modified_base order(4,6,11,12,14,16,26): mod_base = OTHER; note = thymine or uracil substituted with NapdU(5-naphthylmethylaminocarbonyl-dU)
gcgtgtcccattctatccaagacactg

SEQ ID NO: 14 - DNA, 40 bp, synthetic construct
  source 1..40: mol_type = other DNA
  modified_base order(5,10,11,13,18,20,25,26,28,30,40): mod_base = OTHER; note = thymine or uracil substituted with NapdU(5-naphthylmethylaminocarbonyl-dU)
gagatcaagttatagcgtgtcccattctatccaagacact

SEQ ID NO: 15 - DNA, 38 bp, synthetic construct
  source 1..38: mol_type = other DNA
  modified_base order(2,7,8,10,15,17,22,23,25,27,37): mod_base = OTHER; note = thymine or uracil substituted with NapdU(5-naphthylmethylaminocarbonyl-dU)
atcaagttatagcgtgtcccattctatccaagacactg

SEQ ID NO: 16 - DNA, 33 bp, synthetic construct
  source 1..33: mol_type = other DNA
  modified_base order(2,3,5,10,12,17,18,20,22,32): mod_base = OTHER; note = thymine or uracil substituted with NapdU(5-naphthylmethylaminocarbonyl-dU)
gttatagcgtgtcccattctatccaagacactg

SEQ ID NO: 17 - DNA, 30 bp, synthetic construct
  source 1..30: mol_type = other DNA
  modified_base order(2,7,9,14,15,17,19,29): mod_base = OTHER; note = thymine or uracil substituted with NapdU(5-naphthylmethylaminocarbonyl-dU)
atagcgtgtcccattctatccaagacactg

SEQ ID NO: 18 - DNA, 46 bp, synthetic construct
  source 1..46: mol_type = other DNA
  modified_base order(8,13,14,16,21,23,28,29,31,33,43): mod_base = OTHER; note = thymine or uracil substituted with NapdU(5-naphthylmethylaminocarbonyl-dU)
ttcgagatcaagttatagcgtgtcccattctatccaagacactgac

SEQ ID NO: 19 - DNA, 43 bp, synthetic construct; identical to SEQ ID NO: 1
  source 1..43: mol_type = other DNA
  modified_base order(8,13,14,16,21,23,28,29,31,33,43): mod_base = OTHER; note = thymine or uracil substituted with NapdU(5-naphthylmethylaminocarbonyl-dU)

SEQ ID NO: 20 - DNA, 22 bp, synthetic construct
  source 1..22: mol_type = other DNA
ggacgagcagcgtgtcccattc

SEQ ID NO: 21 - DNA, 23 bp, synthetic construct
  source 1..23: mol_type = other DNA
ggacgagcaagtgtcttggatag

SEQ ID NO: 22 - DNA, 26 bp, synthetic construct
  source 1..26: mol_type = other DNA
ggacgagcagagatcaagttatagcg

SEQ ID NO: 23 - DNA, 27 bp, synthetic construct
  source 1..27: mol_type = other DNA
ggacgagcaagtgtcttggatagaatg

SEQ ID NO: 24 - DNA, 43 bp, synthetic construct; identical to SEQ ID NO: 1
  source 1..43: mol_type = other DNA

SEQ ID NO: 25 - DNA, 19 bp, synthetic construct
  source 1..19: mol_type = other DNA
ggccagatcctgtccaagc

SEQ ID NO: 26 - DNA, 21 bp, synthetic construct
  source 1..21: mol_type = other DNA
gtgggtttccaccattagcac

SEQ ID NO: 27 - DNA, 44 bp, synthetic construct
  source 1..44: mol_type = other DNA
  modified_base order(8,13,14,16,21,23,28,29,31,33,43): mod_base = OTHER; note = thymine or uracil substituted with NapdU(5-naphthylmethylaminocarbonyl-dU)
  modified_base 1: mod_base = OTHER; note = Uracil with the -OH group replaced by methoxy at carbon position 2
  modified_base 44: mod_base = OTHER; note = Guanine with the -OH group replaced by methoxy at carbon position 2
ttcgagatcaagttatagcgtgtcccattctatccaagacactg